European Patent Specification EP 3 098 312 B1, published July 19, 2023. Title: Novel fusion and detection method for the same. Applicant: Japanese Foundation for Cancer Research. The sequence listing filed with the application follows.

SEQUENCE LISTING (15 sequences)

SEQ ID NO: 1 - DNA, 5004 bp, Homo sapiens
  CDS (257)..(4846)
gtcgcgggcagctggcgccgcgcggtcctgctctgccggtcgcacggacgcaccggcgggccgccggccggagggacggggcgggagctgggcccgcggacagcgagccggagcgggagccgcgcgtagcgagccgggctccggcgctcgccagtctcccgagcggcgcccgcctcccgccggtgcccgcgccgggccgtggggggcagcatgcccgcgcgcgctgcctgaggacgccgcggcccccgcccccgccatgggcgcccctgcctgcgccctcgcgctctgcgtggccgtggccatcgtggccggcgcctcctcggagtccttggggacggagcagcgcgtcgtggggcgagcggcagaagtcccgggcccagagcccggccagcaggagcagttggtcttcggcagcggggatgctgtggagctgagctgtcccccgcccgggggtggtcccatggggcccactgtctgggtcaaggatggcacagggctggtgccctcggagcgtgtcctggtggggccccagcggctgcaggtgctgaatgcctcccacgaggactccggggcctacagctgccggcagcggctcacgcagcgcgtactgtgccacttcagtgtgcgggtgacagacgctccatcctcgggagatgacgaagacggggaggacgaggctgaggacacaggtgtggacacaggggccccttactggacacggcccgagcggatggacaagaagctgctggccgtgccggccgccaacaccgtccgcttccgctgcccagccgctggcaaccccactccctccatctcctggctgaagaacggcagggagttccgcggcgagcaccgcattggaggcatcaagctgcggcatcagcagtggagcctggtcatggaaagcgtggtgccctcggaccgcggcaactacacctgcgtcgtggagaacaagtttggcagcatccggcagacgtacacgctggacgtgctggagcgctccccgcaccggcccatcctgcaggcggggctgccggccaaccagacggcggtgctgggcagcgacgtggagttccactgcaaggtgtacagtgacgcacagccccacatccagtggctcaagcacgtggaggtgaatggcagcaaggtgggcccggacggcacaccctacgttaccgtgctcaagtcctggatcagtgagagtgtggaggccgacgtgcgcctccgcctggccaatgtgtcggagcgggacgggggcgagtacctctgtcgagccaccaatttcataggcgtggccgagaaggccttttggctgagcgttcacgggccccgagcagccgaggaggagctggtggaggctgacgaggcgggcagtgtgtatgcaggcatcctcagctacggggtgggcttcttcctgttcatcctggtggtggcggctgtgacgctctgccgcctgcgcagcccccccaagaaaggcctgggctcccccaccgtgcacaagatctcccgcttcccgctcaagcgacaggtgtccctggagtccaacgcgtccatgagctccaacacaccactggtgcgcatcgcaaggctgtcctcaggggagggccccacgctggccaatgtctccgagctcgagctgcctgccgaccccaaatgggagctgtctcgggcccggctgaccctgggcaagccccttggggagggctgcttcggccaggtggtcatggcggaggccatcggcattgacaaggaccgggccgccaagcctgtcaccgtagccgtgaagatgctgaaagacgatgccactgacaaggacctgtcggacctggtgtctgagatggagatgatgaagatgatcgggaaacacaaaaacatcatcaacctgctgggcgcctgcacgcagggcgggcccctgtacgtgctggtggagtacgcggccaagggtaacctgcgggagtttctgcgggcgcggcggcccccgggcctggactactccttcgacacctgcaagccgcccgaggagcagctcaccttcaaggacctggtgtcctgtgcctaccaggtggcccggggcatggagtacttggcctcccagaagtgcatccacagggacctggctgcccgcaatgtgctggtgaccgaggacaacgtgatgaagatcgcagacttcgggctggcccgggacgtgcacaacctcgactactacaagaagacgaccaacggccggctgcccgtgaagtggatggcgcctgaggccttgtttgaccgagtctacactcaccagagtgacgtctggtcctttggggtcctgctctgggagatcttcacgctggggggctccccgtaccccggcatccctgtggaggagctcttcaagctgctgaaggagggccaccgcatggacaagcccgccaactgcacacacgacctgtacatgatcatgcgggagtgctggcatgccgcgccctcccagaggcccaccttcaagcagctggtggaggacctggaccgtgtccttaccgtgacgtccaccgacgagtacctggacctgtcggcgcctttcgagcagtactccccgggtggccaggacacccccagctccagctcctcaggggacgactccgtgttaaacagccaacagctcatcaaggaagtggatgccaaaactactcatggaattctacagaaaccagtggaggctgacaccgacctcctgggggatgcaagcccagcctttgggagtggcagctccagcgagtctggcccaggtgccctggctgacctggactgctcaagctcttcccagagcccaggaagttctgagaaccaaatggtgtctccaggaaaagtgtctggcagccctgagcaagccgtggaggaaaaccttagttcctattccttagacagaagagtgacacccgcctctgagaccctagaagacccttgcaggacagagtcccagcacaaagcggagactccgcacggagccgaggaagaatgcaaagcggagactccgcacggagccgaggaggaatgccggcacggtggggtctgtgctcccgcagcagtggccacttcgcctcctggtgcaatccctaaggaagcctgcggaggagcacccctgcagggtctgcctggcgaagccctgggctgccctgcgggtgtgggcacccccgtgccagcagatggcactcagacccttacctgtgcacacacctctgctcctgagagcacagccccaaccaaccacctggtggctggcagggccatgaccctgagtcctcaggaagaagtggctgcaggccaaatggccagctcctcgaggagcggacctgtaaaactagaatttgatgtatctgatggcgccaccagcaaaagggcacccccaccaaggagactgggagagaggtccggcctcaagcctcccttgaggaaagcagcagtgaggcagcaaaaggccccgcaggaggtggaggaggacgacggtaggagcggagcaggagaggacccccccatgccagcttctcggggctcttaccacctcgactgggacaaaatggatgacccaaacttcatcccgttcggaggtgacaccaagtctggttgcagtgaggcccagcccccagaaagccctgagaccaggctgggccagccagcggctgaacagttgcatgctgggcctgccacggaggagccaggtccctgtctgagccagcagctgcattcagcctcagcggaggacacgcctgtggtgcagttggcagccgagaccccaacagcagagagcaaggagagagccttgaactctgccagcacctcgcttcccacaagctgtccaggcagtgagccagtgcccacccatcagcaggggcagcctgccttggagctgaaagaggagagcttcagagaccccgctgaggttctaggcacgggcgcggaggtggattacctggagcagtttggaacttcctcgtttaaggagtcggccttgaggaagcagtccttatacctcaagttcgaccccctcctgagggacagtcctggtagaccagtgcccgtggccaccgagaccagcagcatgcacggtgcaaatgagactccctcaggacgtccgcgggaagccaagcttgtggagttcgatttcttgggagcactggacattcctgtgccaggcccacccccaggtgttcccgcgcctgggggcccacccctgtccaccggacctatagtggacctgctccagtacagccagaaggacctggatgcagtggtaaaggcgacacaggaggagaaccgggagctgaggagcaggtgtgaggagctccacgggaagaacctggaactggggaagatcatggacaggttcgaagaggttgtgtaccaggccatggaggaagttcagaagcagaaggaactttccaaagctgaaatccagaaagttctaaaagaaaaagaccaacttaccacagatctgaactccatggagaagtccttctccgacctcttcaagcgttttgagaaacagaaagaggtgatcgagggctaccgcaagaacgaagagtcactgaagaagtgcgtggaggattacctggcaaggatcacccaggagggccagaggtaccaagccctgaaggcccacgcggaggagaagctgcagctggcaaacgaggagatcgcccaggtccggagcaaggcccaggcggaagcgttggccctccaggccagcctgaggaaggagcagatgcgcatccagtcgctggagaagacagtggagcagaagactaaagagaacgaggagctgaccaggatctgcgacgacctcatctccaagatggagaagatctgacctccacggagccgctgtccccgcccccctgctcccgtctgtctgtcctgtctgattctcttaggtgtcatgttcttttttctgtcttgtcttcaacttttttaaaaactagattgctttgaaaacatgactcaataaaagtttcctttcaatttaaa

SEQ ID NO: 2 - protein, 1529 aa, Homo sapiens [sequence omitted]

SEQ ID NO: 3 - DNA, 3561 bp, Homo sapiens
  CDS (257)..(3403)
gtcgcgggcagctggcgccgcgcggtcctgctctgccggtcgcacggacgcaccggcgggccgccggccggagggacggggcgggagctgggcccgcggacagcgagccggagcgggagccgcgcgtagcgagccgggctccggcgctcgccagtctcccgagcggcgcccgcctcccgccggtgcccgcgccgggccgtggggggcagcatgcccgcgcgcgctgcctgaggacgccgcggcccccgcccccgccatgggcgcccctgcctgcgccctcgcgctctgcgtggccgtggccatcgtggccggcgcctcctcggagtccttggggacggagcagcgcgtcgtggggcgagcggcagaagtcccgggcccagagcccggccagcaggagcagttggtcttcggcagcggggatgctgtggagctgagctgtcccccgcccgggggtggtcccatggggcccactgtctgggtcaaggatggcacagggctggtgccctcggagcgtgtcctggtggggccccagcggctgcaggtgctgaatgcctcccacgaggactccggggcctacagctgccggcagcggctcacgcagcgcgtactgtgccacttcagtgtgcgggtgacagacgctccatcctcgggagatgacgaagacggggaggacgaggctgaggacacaggtgtggacacaggggccccttactggacacggcccgagcggatggacaagaagctgctggccgtgccggccgccaacaccgtccgcttccgctgcccagccgctggcaaccccactccctccatctcctggctgaagaacggcagggagttccgcggcgagcaccgcattggaggcatcaagctgcggcatcagcagtggagcctggtcatggaaagcgtggtgccctcggaccgcggcaactacacctgcgtcgtggagaacaagtttggcagcatccggcagacgtacacgctggacgtgctggagcgctccccgcaccggcccatcctgcaggcggggctgccggccaaccagacggcggtgctgggcagcgacgtggagttccactgcaaggtgtacagtgacgcacagccccacatccagtggctcaagcacgtggaggtgaatggcagcaaggtgggcccggacggcacaccctacgttaccgtgctcaagtcctggatcagtgagagtgtggaggccgacgtgcgcctccgcctggccaatgtgtcggagcgggacgggggcgagtacctctgtcgagccaccaatttcataggcgtggccgagaaggccttttggctgagcgttcacgggccccgagcagccgaggaggagctggtggaggctgacgaggcgggcagtgtgtatgcaggcatcctcagctacggggtgggcttcttcctgttcatcctggtggtggcggctgtgacgctctgccgcctgcgcagcccccccaagaaaggcctgggctcccccaccgtgcacaagatctcccgcttcccgctcaagcgacaggtgtccctggagtccaacgcgtccatgagctccaacacaccactggtgcgcatcgcaaggctgtcctcaggggagggccccacgctggccaatgtctccgagctcgagctgcctgccgaccccaaatgggagctgtctcgggcccggctgaccctgggcaagccccttggggagggctgcttcggccaggtggtcatggcggaggccatcggcattgacaaggaccgggccgccaagcctgtcaccgtagccgtgaagatgctgaaagacgatgccactgacaaggacctgtcggacctggtgtctgagatggagatgatgaagatgatcgggaaacacaaaaacatcatcaacctgctgggcgcctgcacgcagggcgggcccctgtacgtgctggtggagtacgcggccaagggtaacctgcgggagtttctgcgggcgcggcggcccccgggcctggactactccttcgacacctgcaagccgcccgaggagcagctcaccttcaaggacctggtgtcctgtgcctaccaggtggcccggggcatggagtacttggcctcccagaagtgcatccacagggacctggctgcccgcaatgtgctggtgaccgaggacaacgtgatgaagatcgcagacttcgggctggcccgggacgtgcacaacctcgactactacaagaagacgaccaacggccggctgcccgtgaagtggatggcgcctgaggccttgtttgaccgagtctacactcaccagagtgacgtctggtcctttggggtcctgctctgggagatcttcacgctggggggctccccgtaccccggcatccctgtggaggagctcttcaagctgctgaaggagggccaccgcatggacaagcccgccaactgcacacacgacctgtacatgatcatgcgggagtgctggcatgccgcgccctcccagaggcccaccttcaagcagctggtggaggacctggaccgtgtccttaccgtgacgtccaccgacgagtacctggacctgtcggcgcctttcgagcagtactccccgggtggccaggacacccccagctccagctcctcaggggacgactccgtgttaaacagcatgcacggtgcaaatgagactccctcaggacgtccgcgggaagccaagcttgtggagttcgatttcttgggagcactggacattcctgtgccaggcccacccccaggtgttcccgcgcctgggggcccacccctgtccaccggacctatagtggacctgctccagtacagccagaaggacctggatgcagtggtaaaggcgacacaggaggagaaccgggagctgaggagcaggtgtgaggagctccacgggaagaacctggaactggggaagatcatggacaggttcgaagaggttgtgtaccaggccatggaggaagttcagaagcagaaggaactttccaaagctgaaatccagaaagttctaaaagaaaaagaccaacttaccacagatctgaactccatggagaagtccttctccgacctcttcaagcgttttgagaaacagaaagaggtgatcgagggctaccgcaagaacgaagagtcactgaagaagtgcgtggaggattacctggcaaggatcacccaggagggccagaggtaccaagccctgaaggcccacgcggaggagaagctgcagctggcaaacgaggagatcgcccaggtccggagcaaggcccaggcggaagcgttggccctccaggccagcctgaggaaggagcagatgcgcatccagtcgctggagaagacagtggagcagaagactaaagagaacgaggagctgaccaggatctgcgacgacctcatctccaagatggagaagatctgacctccacggagccgctgtccccgcccccctgctcccgtctgtctgtcctgtctgattctcttaggtgtcatgttcttttttctgtcttgtcttcaacttttttaaaaactagattgctttgaaaacatgactcaataaaagtttcctttcaatttaaa

SEQ ID NO: 4 - protein, 1048 aa, Homo sapiens
MGAPACALALCVAVAIVAGASSESLGTEQRVVGRAAEVPGPEPGQQEQLVFGSGDAVELSCPPPGGGPMGPTVWVKDGTGLVPSERVLVGPQRLQVLNASHEDSGAYSCRQRLTQRVLCHFSVRVTDAPSSGDDEDGEDEAEDTGVDTGAPYWTRPERMDKKLLAVPAANTVRFRCPAAGNPTPSISWLKNGREFRGEHRIGGIKLRHQQWSLVMESVVPSDRGNYTCVVENKFGSIRQTYTLDVLERSPHRPILQAGLPANQTAVLGSDVEFHCKVYSDAQPHIQWLKHVEVNGSKVGPDGTPYVTVLKSWISESVEADVRLRLANVSERDGGEYLCRATNFIGVAEKAFWLSVHGPRAAEEELVEADEAGSVYAGILSYGVGFFLFILVVAAVTLCRLRSPPKKGLGSPTVHKISRFPLKRQVSLESNASMSSNTPLVRIARLSSGEGPTLANVSELELPADPKWELSRARLTLGKPLGEGCFGQVVMAEAIGIDKDRAAKPVTVAVKMLKDDATDKDLSDLVSEMEMMKMIGKHKNIINLLGACTQGGPLYVLVEYAAKGNLREFLRARRPPGLDYSFDTCKPPEEQLTFKDLVSCAYQVARGMEYLASQKCIHRDLAARNVLVTEDNVMKIADFGLARDVHNLDYYKKTTNGRLPVKWMAPEALFDRVYTHQSDVWSFGVLLWEIFTLGGSPYPGIPVEELFKLLKEGHRMDKPANCTHDLYMIMRECWHAAPSQRPTFKQLVEDLDRVLTVTSTDEYLDLSAPFEQYSPGGQDTPSSSSSGDDSVLNSMHGANETPSGRPREAKLVEFDFLGALDIPVPGPPPGVPAPGGPPLSTGPIVDLLQYSQKDLDAVVKATQEENRELRSRCEELHGKNLELGKIMDRFEEVVYQAMEEVQKQKELSKAEIQKVLKEKDQLTTDLNSMEKSFSDLFKRFEKQKEVIEGYRKNEESLKKCVEDYLARITQEGQRYQALKAHAEEKLQLANEEIAQVRSKAQAEALALQASLRKEQMRIQSLEKTVEQKTKENEELTRICDDLISKMEKI

SEQ ID NO: 5 - DNA, 3270 bp, Homo sapiens
  CDS (257)..(3112)
gtcgcgggcagctggcgccgcgcggtcctgctctgccggtcgcacggacgcaccggcgggccgccggccggagggacggggcgggagctgggcccgcggacagcgagccggagcgggagccgcgcgtagcgagccgggctccggcgctcgccagtctcccgagcggcgcccgcctcccgccggtgcccgcgccgggccgtggggggcagcatgcccgcgcgcgctgcctgaggacgccgcggcccccgcccccgccatgggcgcccctgcctgcgccctcgcgctctgcgtggccgtggccatcgtggccggcgcctcctcggagtccttggggacggagcagcgcgtcgtggggcgagcggcagaagtcccgggcccagagcccggccagcaggagcagttggtcttcggcagcggggatgctgtggagctgagctgtcccccgcccgggggtggtcccatggggcccactgtctgggtcaaggatggcacagggctggtgccctcggagcgtgtcctggtggggccccagcggctgcaggtgctgaatgcctcccacgaggactccggggcctacagctgccggcagcggctcacgcagcgcgtactgtgccacttcagtgtgcgggtgacagacgctccatcctcgggagatgacgaagacggggaggacgaggctgaggacacaggtgtggacacaggggccccttactggacacggcccgagcggatggacaagaagctgctggccgtgccggccgccaacaccgtccgcttccgctgcccagccgctggcaaccccactccctccatctcctggctgaagaacggcagggagttccgcggcgagcaccgcattggaggcatcaagctgcggcatcagcagtggagcctggtcatggaaagcgtggtgccctcggaccgcggcaactacacctgcgtcgtggagaacaagtttggcagcatccggcagacgtacacgctggacgtgctggagcgctccccgcaccggcccatcctgcaggcggggctgccggccaaccagacggcggtgctgggcagcgacgtggagttccactgcaaggtgtacagtgacgcacagccccacatccagtggctcaagcacgtggaggtgaatggcagcaaggtgggcccggacggcacaccctacgttaccgtgctcaagtcctggatcagtgagagtgtggaggccgacgtgcgcctccgcctggccaatgtgtcggagcgggacgggggcgagtacctctgtcgagccaccaatttcataggcgtggccgagaaggccttttggctgagcgttcacgggccccgagcagccgaggaggagctggtggaggctgacgaggcgggcagtgtgtatgcaggcatcctcagctacggggtgggcttcttcctgttcatcctggtggtggcggctgtgacgctctgccgcctgcgcagcccccccaagaaaggcctgggctcccccaccgtgcacaagatctcccgcttcccgctcaagcgacaggtgtccctggagtccaacgcgtccatgagctccaacacaccactggtgcgcatcgcaaggctgtcctcaggggagggccccacgctggccaatgtctccgagctcgagctgcctgccgaccccaaatgggagctgtctcgggcccggctgaccctgggcaagccccttggggagggctgcttcggccaggtggtcatggcggaggccatcggcattgacaaggaccgggccgccaagcctgtcaccgtagccgtgaagatgctgaaagacgatgccactgacaaggacctgtcggacctggtgtctgagatggagatgatgaagatgatcgggaaacacaaaaacatcatcaacctgctgggcgcctgcacgcagggcgggcccctgtacgtgctggtggagtacgcggccaagggtaacctgcgggagtttctgcgggcgcggcggcccccgggcctggactactccttcgacacctgcaagccgcccgaggagcagctcaccttcaaggacctggtgtcctgtgcctaccaggtggcccggggcatggagtacttggcctcccagaagtgcatccacagggacctggctgcccgcaatgtgctggtgaccgaggacaacgtgatgaagatcgcagacttcgggctggcccgggacgtgcacaacctcgactactacaagaagacgaccaacggccggctgcccgtgaagtggatggcgcctgaggccttgtttgaccgagtctacactcaccagagtgacgtctggtcctttggggtcctgctctgggagatcttcacgctggggggctccccgtaccccggcatccctgtggaggagctcttcaagctgctgaaggagggccaccgcatggacaagcccgccaactgcacacacgacctgtacatgatcatgcgggagtgctggcatgccgcgccctcccagaggcccaccttcaagcagctggtggaggacctggaccgtgtccttaccgtgacgtccaccgacgtaaaggcgacacaggaggagaaccgggagctgaggagcaggtgtgaggagctccacgggaagaacctggaactggggaagatcatggacaggttcgaagaggttgtgtaccaggccatggaggaagttcagaagcagaaggaactttccaaagctgaaatccagaaagttctaaaagaaaaagaccaacttaccacagatctgaactccatggagaagtccttctccgacctcttcaagcgttttgagaaacagaaagaggtgatcgagggctaccgcaagaacgaagagtcactgaagaagtgcgtggaggattacctggcaaggatcacccaggagggccagaggtaccaagccctgaaggcccacgcggaggagaagctgcagctggcaaacgaggagatcgcccaggtccggagcaaggcccaggcggaagcgttggccctccaggccagcctgaggaaggagcagatgcgcatccagtcgctggagaagacagtggagcagaagactaaagagaacgaggagctgaccaggatctgcgacgacctcatctccaagatggagaagatctgacctccacggagccgctgtccccgcccccctgctcccgtctgtctgtcctgtctgattctcttaggtgtcatgttcttttttctgtcttgtcttcaacttttttaaaaactagattgctttgaaaacatgactcaataaaagtttcctttcaatttaaa

SEQ ID NO: 6 - protein, 951 aa, Homo sapiens
MGAPACALALCVAVAIVAGASSESLGTEQRVVGRAAEVPGPEPGQQEQLVFGSGDAVELSCPPPGGGPMGPTVWVKDGTGLVPSERVLVGPQRLQVLNASHEDSGAYSCRQRLTQRVLCHFSVRVTDAPSSGDDEDGEDEAEDTGVDTGAPYWTRPERMDKKLLAVPAANTVRFRCPAAGNPTPSISWLKNGREFRGEHRIGGIKLRHQQWSLVMESVVPSDRGNYTCVVENKFGSIRQTYTLDVLERSPHRPILQAGLPANQTAVLGSDVEFHCKVYSDAQPHIQWLKHVEVNGSKVGPDGTPYVTVLKSWISESVEADVRLRLANVSERDGGEYLCRATNFIGVAEKAFWLSVHGPRAAEEELVEADEAGSVYAGILSYGVGFFLFILVVAAVTLCRLRSPPKKGLGSPTVHKISRFPLKRQVSLESNASMSSNTPLVRIARLSSGEGPTLANVSELELPADPKWELSRARLTLGKPLGEGCFGQVVMAEAIGIDKDRAAKPVTVAVKMLKDDATDKDLSDLVSEMEMMKMIGKHKNIINLLGACTQGGPLYVLVEYAAKGNLREFLRARRPPGLDYSFDTCKPPEEQLTFKDLVSCAYQVARGMEYLASQKCIHRDLAARNVLVTEDNVMKIADFGLARDVHNLDYYKKTTNGRLPVKWMAPEALFDRVYTHQSDVWSFGVLLWEIFTLGGSPYPGIPVEELFKLLKEGHRMDKPANCTHDLYMIMRECWHAAPSQRPTFKQLVEDLDRVLTVTSTDVKATQEENRELRSRCEELHGKNLELGKIMDRFEEVVYQAMEEVQKQKELSKAEIQKVLKEKDQLTTDLNSMEKSFSDLFKRFEKQKEVIEGYRKNEESLKKCVEDYLARITQEGQRYQALKAHAEEKLQLANEEIAQVRSKAQAEALALQASLRKEQMRIQSLEKTVEQKTKENEELTRICDDLISKMEKI

SEQ ID NO: 7 - DNA, 22 bp, Artificial Sequence
  Description of Artificial Sequence: synthetic primer
ctactccttcgacacctgcaag

SEQ ID NO: 8 - DNA, 21 bp, Artificial Sequence
  Description of Artificial Sequence: synthetic primer
ccgtggaggtcagatcttctc

SEQ ID NO: 9 - DNA, 20 bp, Artificial Sequence
  Description of Artificial Sequence: synthetic primer
cactgtctgggtcaaggatg

SEQ ID NO: 10 - DNA, 19 bp, Artificial Sequence
  Description of Artificial Sequence: synthetic primer
tccccgtcttcgtcatctc

SEQ ID NO: 11 - DNA, 22 bp, Artificial Sequence
  Description of Artificial Sequence: synthetic primer
ctgaaattacgggtacctgaag

SEQ ID NO: 12 - DNA, 20 bp, Artificial Sequence
  Description of Artificial Sequence: synthetic primer
tccgttgtaccagccttttc

SEQ ID NO: 13 - DNA, 24 bp, Artificial Sequence
  Description of Artificial Sequence: synthetic primer
agcagctcaccttcaaggacctgg

SEQ ID NO: 14 - DNA, 22 bp, Artificial Sequence
  Description of Artificial Sequence: synthetic primer
gtgaagatgctgaaagacgatg

SEQ ID NO: 15 - DNA, 23 bp, Artificial Sequence
  Description of Artificial Sequence: synthetic primer
ggtcagctcctcgttctctttag